European Patent Specification EP 3 551 758 B1, published May 29, 2024. Title: Codon Optimization. Applicant: Max-Planck-Gesellschaft zur Förderung der Wissenschaften e.V. The sequence listing filed with the application follows.

SEQUENCE LISTING (38 sequences)

SEQ ID NO: 1 - DNA, 18 bp, Artificial Sequence
  Oligonucleotide oHL20
gcctgcttgccgaatatc

SEQ ID NO: 2 - DNA, 61 bp, Artificial Sequence
  Oligonucleotide oJT1
atgcaaaaactcattaactcagtgcaaaactatgcctgggtgtgtaggctggagctgcttc

SEQ ID NO: 3 - DNA, 66 bp, Artificial Sequence
  Oligonucleotide oJT2
ctacagcttgttataaacacgcgctaaacggcccgtgccgctggcgcatatgaatatcctccttag

SEQ ID NO: 4 - DNA, 20 bp, Artificial Sequence
  Oligonucleotide oJT4
gaaaccaggcggattaaacc

SEQ ID NO: 5 - DNA, 31 bp, Artificial Sequence
  Oligonucleotide oJT7
ggatatcatatgcaaaaactcattaactcag

SEQ ID NO: 6 - DNA, 34 bp, Artificial Sequence
  Oligonucleotide oJT8
ggatatcactagtctacagcttgttataaacacg

SEQ ID NO: 7 - DNA, 20 bp, Artificial Sequence
  Oligonucleotide oJT11
tccggcctttattcacattc

SEQ ID NO: 8 - DNA, 20 bp, Artificial Sequence
  Oligonucleotide oJT12
cgtttcagtttgctcatgga

SEQ ID NO: 9 - DNA, 20 bp, Artificial Sequence
  Oligonucleotide oJT13
cctcccattgatctccacat

SEQ ID NO: 10 - DNA, 20 bp, Artificial Sequence
  Oligonucleotide oJT14
ggtcagtgcggttttgctac

SEQ ID NO: 11 - DNA, 20 bp, Artificial Sequence
  Oligonucleotide oJT16
gattggcgatgccataaagt

SEQ ID NO: 12 - DNA, 20 bp, Artificial Sequence
  Oligonucleotide oJT17
attggcgatgccataaagtt

SEQ ID NO: 13 - DNA, 20 bp, Artificial Sequence
  Oligonucleotide oJT21
gttttagagccccatgcgta

SEQ ID NO: 14 - DNA, 20 bp, Artificial Sequence
  Oligonucleotide oJT23
gtttgcgatgccgtacagtt

SEQ ID NO: 15 - DNA, 20 bp, Artificial Sequence
  Oligonucleotide oJT24
gggttggctataccgtacaa

SEQ ID NO: 16 - DNA, 20 bp, Artificial Sequence
  Oligonucleotide oJT27
ccatacagttcggtcagtgc

SEQ ID NO: 17 - DNA, 20 bp, Artificial Sequence
  Oligonucleotide oJT28
tggttgttgttgtggattgg

SEQ ID NO: 18 - DNA, 1176 bp, Artificial Sequence
  Coding sequence for manAwt
atgcaaaaactcattaactcagtgcaaaactatgcctggggaagtaaaactgcgttaacggaactttatggcatcgccaatccgcagcagcagccaatggctgaactctggatgggcgcgcatcccaaaagcagctcgcgaatcaccaccgccaacggcgaaaccgtctccctgcgtgacgccatcgaaaagaataaaaccgccatgctgggcgaagcggtagccaaccgtttcggcgaactgccgtttctgtttaaagtactgtgcgccgcacaaccgctctctattcaggtgcacccgaataaacgcaactccgaaatcggtttcgcgaaagaaaatgcggcgggtatccccatggatgccgcagagcggaactataaagatcctaaccataaaccagagctggtttttgccctgacgcctttcctggcgatgaacgcgttccgcgaattttctgacattgtctctttactgcaacctgtcgccggcgcgcattccgctatcgcccactttttgcaggtgccgaatgctgaacgtctgagccagcttttcgccagcctgttgaatatgcaaggcgaagaaaaatcccgcgcgttagccgtactcaaagcggcgcttaacagccagcaaggcgaaccgtggcaaacgatccgcgtgatttcagagtattatcctgacgacagcgggcttttctctcctttgttgctgaatgtggtcaaactgaatcccggcgaggcgatgttcctgtttgctgaaacgcctcatgcttatctgcagggcgttgcgctggaagtcatggcgaactccgataacgttctgcgcgctggccttacgccaaaatatatcgacatccctgagctggtcgcgaacgtgaagttcgaacctaagcctgccggcgagttgctgactgccccggtgaaaagcggcgcggagctggacttcccaattccggttgacgattttgctttttcactgcacgacctggcgcttcaggagacgagcatcggccaacacagcgccgcgattctgttctgcgttgagggtgaggcggtgttacgtaaagatgaacagcgtctggtactgaagccgggtgaatctgcctttatcggcgcggatgagtctccggttaacgccagcggcacgggccgtttagcgcgtgtttataacaagctgtag

SEQ ID NO: 19 - DNA, 1176 bp, Artificial Sequence
  Coding sequence for manA1
atgcagaaactgattaatagcgtgcagaattatgcatggggatcgaaaaccgcactgaccgaactgtatggtattgcaaatccgcagcagcagccaatggcagaactgtggatgggtgcacatccgaaaagcagctcccgaattaccaccgcaaatggtgaaaccgttagcctgcgtgatgcaatcgaaaaaaacaaaaccgccatgctgggtgaagcagttgcaaatcgttttggtgaactgccgtttctgtttaaagttctgtgtgcagcacagccgctgagcattcaggttcatccgaataaacgtaatagcgaaattggctttgccaaagaaaatgcagcaggtattcccatggatgcagcagaacgtaactataaagatccgaatcataaaccagaactggtttttgcactgaccccgtttctggcaatgaatgcatttcgtgaatttagcgatattgtgagcctgctgcagccggttgccggtgcccatagcgcaattgcacattttctgcaggttccgaatgccgaacgtctgagccagctgtttgcaagcctgctgaatatgcagggtgaagaaaaaagccgtgcactggcagttctgaaagcagcactgaatagccagcagggcgaaccgtggcagaccattcgtgttattagcgaatattatccggatgatagcggtctttttagccctctgctgctgaatgttgttaaactgaatccgggtgaagccatgtttctgttcgcagaaacaccgcatgcttatctgcagggtgttgcactggaagttatggcaaatagcgataatgttctgcgtgcaggtctgaccccgaaatacattgatattccagaactggttgccaacgtgaaatttgaaccgaaaccggcaggcgaactgctgaccgcaccggttaaaagcggtgcagaactggattttccgattccggtggatgattttgcatttagtttgcatgatctggcactgcaagaaaccagcattggtcagcatagcgcagcaattctgttttgtgttgaaggtgaagccgttctgcgtaaagatgaacagcgtctggttctgaaacctggtgaaagcgcatttattggtgcagatgaaagtccggttaatgcaagcggcaccggtcgtctggcacgtgtttataacaaactgtaa

SEQ ID NO: 20 - DNA, 1176 bp, Artificial Sequence
  Coding sequence for manA2
atgcagaaactgattaatagcgtgcagaattatgcatggggtagcaaaaccgcactgaccgaactgtatggtattgcaaatccgcagcagcagccgatggcagaactgtggatgggtgcacatccgaaaagcagcagtcgtattaccaccgcaaatggtgaaaccgttagcctgcgtgatgcaatcgaaaaaaacaaaaccgccatgctgggtgaagcagttgcaaatcgttttggtgaactgccgtttctgtttaaagttctgtgtgcagcacagccgctgagcattcaggttcatccgaataaacgtaatagcgaaattggctttgccaaagaaaatgcagcaggtattccgatggatgcagcagaacgtaactataaagatccgaatcataaaccggaactggtttttgcactgaccccgtttctggcaatgaatgcatttcgtgaatttagcgatattgtgagcctgctgcagccggttgccggtgcacatagcgcaattgcacattttctgcaggttccgaatgcagaacgtctgagccagctgtttgcaagcctgctgaatatgcagggtgaagaaaaaagccgtgcactggcagttctgaaagcagcactgaatagccagcagggcgaaccgtggcagaccattcgtgttattagcgaatattatccggatgatagcggtctgtttagccctctgctgctgaatgttgttaaactgaatccgggtgaagccatgtttctgttcgcagaaacaccgcatgcatatctgcagggtgttgcactggaagttatggcaaatagcgataatgttctgcgtgcaggtctgaccccgaaatacattgatattccagaactggttgccaacgtgaaatttgaaccgaaaccggcaggcgaactgctgaccgcaccggttaaaagcggtgcagaactggattttccgattccggtggatgattttgcatttagtctgcatgatctggcactgcaagaaaccagcattggtcagcatagcgcagcaattctgttttgtgttgaaggtgaagccgttctgcgtaaagatgaacagcgtctggttctgaaacctggtgaaagcgcatttattggtgcagatgaaagtccggttaatgcaagcggcaccggtcgtctggcacgtgtttataacaaactgtaa

SEQ ID NO: 21 - DNA, 1176 bp, Artificial Sequence
  Coding sequence for manA3
atgcaaaaactcattaactcagtgcaaaactatgcctggggaagtaaaactgcgttaacggaactttatggcatcgccaatcctcagcagcagccaatggctgaactctggatgggcgcgcatcccaaaagctcatcgcgaatcacgaccgcgaatggtgaaaccgttagcctgcgtgatgcaatcgaaaaaaacaaaaccgccatgctgggtgaagcagttgcaaatcgttttggtgaactgccgtttctgtttaaagttctgtgtgcagcacagccgctgagcattcaggttcatccgaataaacgtaatagcgaaattggctttgccaaagaaaatgcagcaggtattccgatggatgcagcagaacgtaactataaagatccgaatcataaaccagaactggtttttgcactgaccccgtttctggcaatgaatgcatttcgtgaatttagcgatattgtgagcctgctgcagccggttgccggtgcccatagcgcaattgcacattttctgcaggttccgaatgccgaacgtctgagccagctgtttgcaagcctgctgaatatgcagggtgaagaaaaaagccgtgcactggcagttctgaaagcagcactgaatagccagcagggcgaaccgtggcagaccattcgtgttattagcgaatattatccggatgatagcggtctttttagccctctgctgctgaatgttgttaaactgaatccgggtgaagccatgtttctgttcgcagaaacaccgcatgcttatctgcagggtgttgcactggaagttatggcaaatagcgataatgttctgcgtgcaggtctgaccccgaaatacattgatattccagaactggttgccaacgtgaaatttgaaccgaaaccggcaggcgaactgctgaccgcaccggttaaaagcggtgcagaactggattttccgattccggtggatgattttgcatttagtttgcatgatctggcactgcaagaaaccagcattggtcagcatagcgcagcaattctgttttgtgttgaaggtgaagccgttctgcgtaaagatgaacagcgtctggttctgaaacctggtgaaagcgcatttattggtgcagatgaaagtccggttaatgcaagcggcaccggtcgtctggcacgtgtttataacaaactgtaa

SEQ ID NO: 22 - DNA, 1176 bp, Artificial Sequence
  Coding sequence for manA4a
atgcaaaagctaataaattccgtccaaaattatgcctggggatccaagaccgccctaaccgagctatatggaatagccaatccacaacaacaaccaatggccgagctatggatgggagcccatccaaagtcctcctcccggataaccaccgccaatggagagaccgtctccctacgggatgccatagagaagaataagaccgccatgctaggagaggccgtcgccaatcggtttggagagctaccatttctatttaaggtcctatgtgccgcccaaccactatccatacaagtccatccaaataagcggaattccgagataggatttgccaaggagaatgccgccggaataccaatggatgccgccgagcggaattataaggatccaaatcataagccagagctagtctttgccctaaccccatttctagccatgaatgcctttcgggagttttccgatatagtctccctactacaaccagtcgccggagcccattccgccatagcccattttctacaagtcccaaatgccgagcggctatcccaactatttgcctccctactaaatatgcaaggagaggagaagtcccgggccctagccgtcctaaaggccgccctaaattcccaacaaggagagccatggcaaaccatacgggtcatatccgagtattatccagatgattccggactattttccccactactactaaatgtcgtcaagctaaatccaggagaggccatgtttctatttgccgagaccccacatgcctatctacaaggagtcgccctagaggtcatggccaattccgataatgtcctacgggccggactaaccccaaagtatatagatataccagagctagtcgccaatgtcaagtttgagccaaagccagccggagagctactaaccgccccagtcaagtccggagccgagctagattttccaataccagtcgatgattttgccttttccctacatgatctagccctacaagagacctccataggacaacattccgccgccatactattttgtgtcgagggagaggccgtcctacggaaggatgagcaacggctagtcctaaagccaggagagtccgcctttataggagccgatgagtccccagtcaatgcctccggaaccggacggctagcccgggtctataataagctatag

SEQ ID NO: 23 - DNA, 1176 bp, Artificial Sequence
  Coding sequence for manA5
atgcagaaactgatcaactcagttcagaactacgcatggggctcaaaaacggcactgacggaactgtacggcatcgcaaacccccagcagcagcccatggcagaactgtggatgggcgcacaccccaaatcatcatcacgaatcacgacggcaaacggcgaaacggtttcactgcgagacgcaatcgaaaaaaacaaaacggcaatgctgggcgaagcagttgcaaaccgattcggcgaactgcccttcctgttcaaagttctgtgcgcagcacagcccctgtcaatccaggttcaccccaacaaacgaaactcagaaatcggcttcgcaaaagaaaacgcagcaggcatccccatggacgcagcagaacgaaactacaaagaccccaaccacaaacccgaactggttttcgcactgacgcccttcctggcaatgaacgcattccgagaattctcagacatcgtttcactgctgcagcccgttgcaggcgcacactcagcaatcgcacacttcctgcaggttcccaacgcagaacgactgtcacagctgttcgcatcactgctgaacatgcagggcgaagaaaaatcacgagcactggcagttctgaaagcagcactgaactcacagcagggcgaaccctggcagacgatccgagttatctcagaatactaccccgacgactcaggcctgttctcacccctgctgctgaacgttgttaaactgaaccccggcgaagcaatgttcctgttcgcagaaacgccccacgcatacctgcagggcgttgcactggaagttatggcaaactcagacaacgttctgcgagcaggcctgacgcccaaatacatcgacatccccgaactggttgcaaacgttaaattcgaacccaaacccgcaggcgaactgctgacggcacccgttaaatcaggcgcagaactggacttccccatccccgttgacgacttcgcattctcactgcacgacctggcactgcaggaaacgtcaatcggccagcactcagcagcaatcctgttctgcgttgaaggcgaagcagttctgcgaaaagacgaacagcgactggttctgaaacccggcgaatcagcattcatcggcgcagacgaatcacccgttaacgcatcaggcacgggccgactggcacgagtttacaacaaactgtag

SEQ ID NO: 24 - DNA, 1176 bp, Artificial Sequence
  Coding sequence for manA6
atgcaaaagctcataaactctgtgcaaaattatgcatggggtagcaagactgctctaacagaattgtacggtatagccaacccgcaacagcaacctatggccgaactatggatgggtgctcacccaaagtcgagctcccggataactaccgccaacggagagaccgtctcacttagagatgcgattgagaagaataaaaccgccatgcttggggaggcggttgccaatcggtttggtgagttaccatttctctttaaagtattatgtgccgcccagccactctcgatacaggtgcatccgaataaaagaaatagtgagataggatttgccaaagaaaacgcagcagggataccaatggacgccgcagagcggaattataaagacccaaatcacaagcccgagttagtgttcgccttaaccccatttctagccatgaacgcattcagagagttcagtgatatagtcagcctactacagccagtcgctggagcccatagcgctatcgcccactttcttcaggtgccaaacgccgaacggctcagccaactttttgcgagtctattaaatatgcagggtgaggaaaagtcgagggcacttgccgtgctaaaggcagccctaaattcccagcaaggagagccatggcaaactatacgcgtcatatcggaatactatcctgacgactccgggctgtttagtccgctactacttaacgtcgttaaactaaatccgggcgaagcgatgtttttatttgctgaaacccctcacgcctatcttcagggtgtcgccctcgaagtgatggctaattcagataatgtcttacgggccggtctcacaccaaagtatatagacatcccagaattagtcgccaacgtgaagttcgaaccaaagccggccggcgagctcttgaccgccccagtcaagagcggtgctgaactagattttccaataccagtcgacgacttcgccttttccctccatgaccttgcccttcaggagacctccataggacagcatagcgccgcaatactattctgcgtcgaaggagaagccgtgctccggaaggatgagcaacggcttgtgttgaagccaggagagagcgcattcataggagccgatgagagtccggttaatgcttccggtaccggtagactagccagggtgtataacaaactgtag

SEQ ID NO: 25 - DNA, 1176 bp, Artificial Sequence
  Coding sequence for manA7
atgcagaaactgatcaactctgttcagaactacgcatggggctctaaaacggcactgacggaactgtacggcatcgcaaaccctcagcagcagcctatggcagaactgtggatgggcgcacaccctaaatcttcttctcgaatcacgacggcaaacggcgaaacggtttctctgcgagacgcaatcgaaaaaaacaaaacggcaatgctgggcgaagcagttgcaaaccgattcggcgaactgcctttcctgttcaaagttctgtgcgcagcacagcctctgtctatccaggttcaccctaacaaacgaaactctgaaatcggcttcgcaaaagaaaacgcagcaggcatccctatggacgcagcagaacgaaactacaaagaccctaaccacaaacctgaactggttttcgcactgacgcctttcctggcaatgaacgcattccgagaattctctgacatcgtttctctgctgcagcctgttgcaggcgcacactctgcaatcgcacacttcctgcaggttcctaacgcagaacgactgtctcagctgttcgcatctctgctgaacatgcagggcgaagaaaaatctcgagcactggcagttctgaaagcagcactgaactctcagcagggcgaaccttggcagacgatccgagttatctctgaatactaccctgacgactctggcctgttctctcctctgctgctgaacgttgttaaactgaaccctggcgaagcaatgttcctgttcgcagaaacgcctcacgcatacctgcagggcgttgcactggaagttatggcaaactctgacaacgttctgcgagcaggcctgacgcctaaatacatcgacatccctgaactggttgcaaacgttaaattcgaacctaaacctgcaggcgaactgctgacggcacctgttaaatctggcgcagaactggacttccctatccctgttgacgacttcgcattctctctgcacgacctggcactgcaggaaacgtctatcggccagcactctgcagcaatcctgttctgcgttgaaggcgaagcagttctgcgaaaagacgaacagcgactggttctgaaacctggcgaatctgcattcatcggcgcagacgaatctcctgttaacgcatctggcacgggccgactggcacgagtttacaacaaactgtaa

SEQ ID NO: 26 - DNA, 1176 bp, Artificial Sequence
  Coding sequence for manA8
atgcaaaaactcattaactcagtgcaaaactatgcctggggaagtaaaactgcgttaacggaactttatggcatcgccaatcctcagcagcagccaatggctgaactctggatgggcgcgcatcccaaaagctcatcgcgaatcacgaccgcaaacggcgaaacggtttcactgcgagacgcaatcgaaaaaaacaaaacggcaatgctgggcgaagcagttgcaaaccgattcggcgaactgcccttcctgttcaaagttctgtgcgcagcacagcccctgtcaatccaggttcaccccaacaaacgaaactcagaaatcggcttcgcaaaagaaaacgcagcaggcatccccatggacgcagcagaacgaaactacaaagaccccaaccacaaacccgaactggttttcgcactgacgcccttcctggcaatgaacgcattccgagaattctcagacatcgtttcactgctgcagcccgttgcaggcgcacactcagcaatcgcacacttcctgcaggttcccaacgcagaacgactgtcacagctgttcgcatcactgctgaacatgcagggcgaagaaaaatcacgagcactggcagttctgaaagcagcactgaactcacagcagggcgaaccctggcagacgatccgagttatctcagaatactaccccgacgactcaggcctgttctcacccctgctgctgaacgttgttaaactgaaccccggcgaagcaatgttcctgttcgcagaaacgccccacgcatacctgcagggcgttgcactggaagttatggcaaactcagacaacgttctgcgagcaggcctgacgcccaaatacatcgacatccccgaactggttgcaaacgttaaattcgaacccaaacccgcaggcgaactgctgacggcacccgttaaatcaggcgcagaactggacttccccatccccgttgacgacttcgcattctcactgcacgacctggcactgcaggaaacgtcaatcggccagcactcagcagcaatcctgttctgcgttgaaggcgaagcagttctgcgaaaagacgaacagcgactggttctgaaacccggcgaatcagcattcatcggcgcagacgaatcacccgttaacgcatcaggcacgggccgactggcacgagtttacaacaaactgtag

SEQ ID NO: 27 - DNA, 1176 bp, Artificial Sequence
  Coding sequence for manA9
atgcaaaaactcattaactcagtgcaaaactatgcctggggaagtaaaactgcgttaacggaactttatggcatcgccaatcctcagcagcagccaatggctgaactctggatgggcgcgcatcccaaaagctcatcgcgaatcacgaccgccaacggagagaccgtctcacttagagatgcgattgagaagaataaaaccgccatgcttggggaggcggttgccaatcggtttggtgagttaccatttctctttaaagtattatgtgccgcccagccactctcgatacaggtgcatccgaataaaagaaatagtgagataggatttgccaaagaaaacgcagcagggataccaatggacgccgcagagcggaattataaagacccaaatcacaagcccgagttagtgttcgccttaaccccatttctagccatgaacgcattcagagagttcagtgatatagtcagcctactacagccagtcgctggagcccatagcgctatcgcccactttcttcaggtgccaaacgccgaacggctcagccaactttttgcgagtctattaaatatgcagggtgaggaaaagtcgagggcacttgccgtgctaaaggcagccctaaattcccagcaaggagagccatggcaaactatacgcgtcatatcggaatactatcctgacgactccgggctgtttagtccgctactacttaacgtcgttaaactaaatccgggcgaagcgatgtttttatttgctgaaacccctcacgcctatcttcagggtgtcgccctcgaagtgatggctaattcagataatgtcttacgggccggtctcacaccaaagtatatagacatcccagaattagtcgccaacgtgaagttcgaaccaaagccggccggcgagctcttgaccgccccagtcaagagcggtgctgaactagattttccaataccagtcgacgacttcgccttttccctccatgaccttgcccttcaggagacctccataggacagcatagcgccgcaatactattctgcgtcgaaggagaagccgtgctccggaaggatgagcaacggcttgtgttgaagccaggagagagcgcattcataggagccgatgagagtccggttaatgcttccggtaccggtagactagccagggtgtataacaaactgtag

SEQ ID NO: 28 - DNA, 1176 bp, Artificial Sequence
  Coding sequence for manA10
atgcaaaaactcattaactcagtgcaaaactatgcctggggaagtaaaactgcgttaacggaactttatggcatcgccaatcctcagcagcagccaatggctgaactctggatgggcgcgcatcccaaaagctcatcgcgaatcacgaccgcaaacggcgaaacggtttctctgcgagacgcaatcgaaaaaaacaaaacggcaatgctgggcgaagcagttgcaaaccgattcggcgaactgcctttcctgttcaaagttctgtgcgcagcacagcctctgtctatccaggttcaccctaacaaacgaaactctgaaatcggcttcgcaaaagaaaacgcagcaggcatccctatggacgcagcagaacgaaactacaaagaccctaaccacaaacctgaactggttttcgcactgacgcctttcctggcaatgaacgcattccgagaattctctgacatcgtttctctgctgcagcctgttgcaggcgcacactctgcaatcgcacacttcctgcaggttcctaacgcagaacgactgtctcagctgttcgcatctctgctgaacatgcagggcgaagaaaaatctcgagcactggcagttctgaaagcagcactgaactctcagcagggcgaaccttggcagacgatccgagttatctctgaatactaccctgacgactctggcctgttctctcctctgctgctgaacgttgttaaactgaaccctggcgaagcaatgttcctgttcgcagaaacgcctcacgcatacctgcagggcgttgcactggaagttatggcaaactctgacaacgttctgcgagcaggcctgacgcctaaatacatcgacatccctgaactggttgcaaacgttaaattcgaacctaaacctgcaggcgaactgctgacggcacctgttaaatctggcgcagaactggacttccctatccctgttgacgacttcgcattctctctgcacgacctggcactgcaggaaacgtctatcggccagcactctgcagcaatcctgttctgcgttgaaggcgaagcagttctgcgaaaagacgaacagcgactggttctgaaacctggcgaatctgcattcatcggcgcagacgaatctcctgttaacgcatctggcacgggccgactggcacgagtttacaacaaactgtaa

SEQ ID NO: 29 - DNA, 1176 bp, Artificial Sequence; identical to SEQ ID NO: 22
  Coding sequence for manA4

SEQ ID NO: 30 - DNA, 1176 bp, Artificial Sequence; identical to SEQ ID NO: 22
  Coding sequence for manA4b

SEQ ID NO: 31 - DNA, 1176 bp, Artificial Sequence; identical to SEQ ID NO: 22
  Coding sequence for manA4c

SEQ ID NO: 32 - DNA, 75 bp, Artificial Sequence
  5' utr
aggttacttcatgcgggtttcttggtttaatacctcccattgatctccacattgaaacagggcttgatacatatg

SEQ ID NO: 33 - DNA, 31 bp, Artificial Sequence
  5' utr promoter
ctccacattgaaacagggcttgatacatatg

SEQ ID NO: 34 - DNA, 1158 bp, Artificial Sequence
  Coding sequence for ova_origOptAcc
atgggctcaatcggcgcagcatcaatggaattctgcttcgacgttttcaaagaactgaaagttcaccacgcaaacgaaaacatcttctactgccccatcgcaatcatgtcagcactggcaatggtttacctgggcgcaaaagactcaacgcgaacgcagatcaacaaagttgttcgattcgacaaactgcccggcttcggcgactcaatcgaagcacagtgcggcacgtcagttaacgttcactcatcactgcgagacatcctgaaccagatcacgaaacccaacgacgtttactcattctcactggcatcacgactgtacgcagaagaacgataccccatcctgcccgaatacctgcagtgcgttaaagaactgtaccgaggcggcctggaacccatcaacttccagacggcagcagaccaggcacgagaactgatcaactcatgggttgaatcacagacgaacggcatcatccgaaacgttctgcagccctcatcagttgactcacagacggcaatggttctggttaacgcaatcgttttcaaaggcctgtgggaaaaaacgttcaaagacgaagacacgcaggcaatgcccttccgagttacggaacaggaatcaaaacccgttcagatgatgtaccagatcggcctgttccgagttgcatcaatggcatcagaaaaaatgaaaatcctggaactgcccttcgcatcaggcacgatgtcaatgctggttctgctgcccgacgaagtttcaggcctggaacagctggaatcaatcatcaacttcgaaaaactgacggaatggacgtcatcaaacgttatggaagaacgaaaaatcaaagtttacctgccccgaatgaaaatggaagaaaaatacaacctgacgtcagttctgatggcaatgggcatcacggacgttttctcatcatcagcaaacctgtcaggcatctcatcagcagaatcactgaaaatctcacaggcagttcacgcagcacacgcagaaatcaacgaagcaggccgagaagttgttggctcagcagaagcaggcgttgacgcagcatcagtttcagaagaattccgagcagaccaccccttcctgttctgcatcaaacacatcgcaacgaacgcagttctgttcttcggccgatgcgtttcaccc

SEQ ID NO: 35 - DNA, 1158 bp, Artificial Sequence
  Coding sequence for ovasyn
atgggcagcattggagcagcttccatggaattctgcttcgacgtgttcaaagagctgaaagtccaccacgctaacgaaaacatcttctattgtccgatcgccattatgagcgccctggcaatggtttatctgggtgccaaagattctacccgtacacagattaacaaagtggtccgcttcgacaaactgcctggttttggtgatagcatcgaggcacagtgtggtacaagtgtgaacgtccattctagcctgcgtgatattctgaatcagattacgaaaccgaacgacgtgtattccttttcactggccagtcgtctgtatgccgaagaacgttatcctattctgccggagtatctgcaatgcgtgaaagaactgtatcgtggcggtctggaaccaatcaattttcaaacggccgctgatcaagcacgtgaactgattaacagttgggtggaaagtcagaccaatggcattatccgtaatgtgctgcagcctagcagtgttgattctcagacggcaatggtcctggttaacgctattgtgtttaaaggcctgtgggagaaaacattcaaagacgaggatacccaagcaatgcctttccgtgttaccgagcaggaaagcaaacctgttcagatgatgtatcaaattgggctgttccgtgtggcaagcatggcatccgaaaaaatgaaaatcctggagctgccttttgctagtggtacaatgagcatgctggttctgctgccagatgaagtttcaggtctggagcaactggaaagcatcatcaacttcgagaaactgaccgagtggacctcttctaacgtgatggaggagcgtaaaatcaaagtctatctgcctcgtatgaaaatggaagagaaatataacctgacctccgtgctgatggctatggggattactgacgtgtttagcagtagcgccaatctgagtgggatttcaagcgctgagtctctgaaaatctctcaggccgttcatgccgctcatgccgaaatcaatgaagccggtcgtgaagtcgtgggaagtgctgaagccggggtggatgccgcttctgttagcgaagaatttcgtgccgatcacccgtttctgttctgtatcaaacacattgctaccaacgccgtactgttttttggacgctgtgtgagcccg

SEQ ID NO: 36 - DNA, 1158 bp, Artificial Sequence
  Coding sequence for ova_orig5050
atgggctcaatcggcgctgcttccatggaattttgttttgacgtattcaaagaactgaaagttcaccatgccaacgaaaacatcttctattgtccaatcgctatcatgtccgccctggcaatggtatacctgggcgccaaagactcaacaaggacgcaaatcaataaggtggttcgatttgacaagctgcccggcttcggtgactcgatcgaggcgcagtgcgggacctcagttaatgttcactcatcactgcgcgatattctgaatcagattacgaaacctaatgatgtgtactcgttctcattggcatctcgactatacgcagaagagcgctatccgatcttacccgagtacttgcaatgcgtgaaagagctttaccgagggggcctggaaccgatcaattttcagactgctgccgaccaagctcgagagcttattaactcttgggttgaatcacaaacaaacggaatcatccgtaatgtactgcagccctcttcagtggactcacaaactgccatggtcttggtaaatgcgatcgtatttaaaggtttgtgggagaagactttcaaagacgaagacacacaagctatgccgttccgagttacggaacaagagtcaaagcctgttcaaatgatgtatcaaatcggcttattccgagtagcatcgatggcaagcgaaaaaatgaagatcctggagctgcctttcgcatcagggacgatgtcaatgttggtattactccctgatgaagtctcaggtctggaacagctggagtctattatcaacttcgaaaaactgaccgaatggacttcatcgaatgttatggaagaacgcaaaatcaaggtgtacttgccccgaatgaagatggaggaaaaatataatctgactagtgttctgatggcgatggggatcacagacgtattttcatcgtctgctaatttgagtggaatctcatcggctgagtcgctaaagatctcacaagctgtgcacgcggcacatgctgagatcaacgaggcggggcgagaagtagttggtagtgctgaagcgggggttgacgcagcctcagtatcggaggaattccgtgccgatcaccccttcttattttgcatcaagcacattgcaacaaacgccgtcttattctttgggcgatgtgtttcccca

SEQ ID NO: 37 - DNA, 1158 bp, Artificial Sequence
  Coding sequence for ova_orig
atgggctccatcggcgcagcaagcatggaattttgttttgatgtattcaaggagctcaaagtccaccatgccaatgagaacatcttctactgccccattgccatcatgtcagctctagccatggtatacctgggtgcaaaagacagcaccaggacacagataaataaggttgttcgctttgataaacttccaggattcggagacagtattgaagctcagtgtggcacatctgtaaacgttcactcttcacttagagacatcctcaaccaaatcaccaaaccaaatgatgtttattcgttcagccttgccagtagactttatgctgaagagagatacccaatcctgccagaatacttgcagtgtgtgaaggaactgtatagaggaggcttggaacctatcaactttcaaacagctgcagatcaagccagagagctcatcaattcctgggtagaaagtcagacaaatggaattatcagaaatgtccttcagccaagctccgtggattctcaaactgcaatggttctggttaatgccattgtcttcaaaggactgtgggagaaaacatttaaggatgaagacacacaagcaatgcctttcagagtgactgagcaagaaagcaaacctgtgcagatgatgtaccagattggtttatttagagtggcatcaatggcttctgagaaaatgaagatcctggagcttccatttgccagtgggacaatgagcatgttggtgctgttgcctgatgaagtctcaggccttgagcagcttgagagtataatcaactttgaaaaactgactgaatggaccagttctaatgttatggaagagaggaagatcaaagtgtacttacctcgcatgaagatggaggaaaaatacaacctcacatctgtcttaatggctatgggcattactgacgtgtttagctcttcagccaatctgtctggcatctcctcagcagagagcctgaagatatctcaagctgtccatgcagcacatgcagaaatcaatgaagcaggcagagaggtggtagggtcagcagaggctggagtggatgctgcaagcgtctctgaagaatttagggctgaccatccattcctcttctgtatcaagcacatcgcaaccaacgccgttctcttctttggcagatgtgtttcccct

SEQ ID NO: 38 - DNA, 1158 bp, Artificial Sequence
  Coding sequence for ova_origOptSpeed
atgggaagcataggcgcagcttccatggaattttgcttcgacgtatttaaggagctaaaggtccatcatgccaatgagaatatattttattgtccaatagccataatgtccgccctagccatggtctatctaggagccaaggattccacccggacccaaataaataaggtcgtccggtttgataagctaccaggatttggagattccatagaggcccaatgtggaacctccgtcaatgtccattcctccctacgggatatactaaatcaaataaccaagccaaatgatgtctattccttttccctagcctcccggctatatgccgaggagcggtatccaatactaccagagtatctacaatgtgtcaaggagctatatcggggaggactagagccaataaattttcaaaccgccgccgatcaagcccgggagctaataaattcctgggtcgagtcccaaaccaatggaataatacggaatgtcctacaaccatcctccgtcgattcccaaaccgccatggtcctagtcaatgccatagtctttaagggactatgggagaagacctttaaggatgaggatacccaagccatgccatttcgggtcaccgagcaagagtccaagccagtccaaatgatgtatcaaataggactatttcgggtcgcctccatggcctccgagaagatgaagatactagagctaccatttgcctccggaaccatgtccatgctagtcctactaccagatgaggtctccggactagagcaactagagtccataataaattttgagaagctaaccgagtggacctcctccaatgtcatggaggagcggaagataaaggtctatctaccacggatgaagatggaggagaagtataatctaacctccgtcctaatggccatgggaataaccgatgtcttttcctcctccgccaatctatccggaatatcctccgccgagtccctaaagatatcccaagccgtccatgccgcccatgccgagataaatgaggccggacgggaggtcgtcggatccgccgaggccggagtcgatgccgcctccgtctccgaggagtttcgggccgatcatccatttctattttgtataaagcatatagccaccaatgccgtcctattttttggacggtgtgtctcccca